European Patent Specification EP 4 405 750 B1, published April 22, 2026. Title: CURABLE RESIN COMPOSITIONS. Applicant: Illumina Cambridge Limited. Application EP. The sequence listing filed with the application follows.

SEQUENCE LISTING (8 sequences)

SEQ ID NO: 1 - DNA, 29 bp, synthetic construct
  source 1..29: mol_type = other DNA
  modified_base 23: mod_base = OTHER; note = uracil
aatgatacggcgaccaccgagatctacac

SEQ ID NO: 2 - DNA, 24 bp, synthetic construct
  source 1..24: mol_type = other DNA
  modified_base 22: mod_base = OTHER; note = 8-oxoguanine
caagcagaagacggcatacganat

SEQ ID NO: 3 - DNA, 24 bp, synthetic construct
  source 1..24: mol_type = other DNA
  modified_base 20: mod_base = OTHER; note = 8-oxoguanine
caagcagaagacggcatacnagat

SEQ ID NO: 4 - DNA, 29 bp, synthetic construct
  source 1..29: mol_type = other DNA
  modified_base 23: mod_base = OTHER; note = allyl-T
aatgatacggcgaccaccgaganctacac

SEQ ID NO: 5 - DNA, 35 bp, synthetic construct
  source 1..35: mol_type = other DNA
gctggcacgtccgaacgcttcgttaatccgttgag

SEQ ID NO: 6 - DNA, 35 bp, synthetic construct
  source 1..35: mol_type = other DNA
cgtcgtctgccatggcgcttcggtggatatgaact

SEQ ID NO: 7 - DNA, 35 bp, synthetic construct
  source 1..35: mol_type = other DNA
acggccgctaatatcaacgcgtcgaatccgcaact

SEQ ID NO: 8 - DNA, 34 bp, synthetic construct
  source 1..34: mol_type = other DNA
gccgcgttacgttagccggactattcgatgcagc